European Patent Application EP 4 438 051 A1, published October 2, 2024. Title: Microbiome-based composition for preventing and treating multidrug resistant bacterial infections. Applicant: 주식회사 바이오미. Application EP 24159416.7, filed February 23, 2024. The sequence listing filed with the application follows.

SEQUENCE LISTING (4 sequences)

SEQ ID NO: 1 - DNA, 1220 bp, unidentified
  source 1..1220: mol_type = genomic DNA
ggaggggcggcgtgcttacacgtgggagtctgacgaaacaccttatttgattttcttcggaactgaagatttggtgattgagtggcggacgggtgagtaacgcgtgggtaacctgccctgtacagggggataacagtcagaaatgactgctaataccgcataagaccacagcaccgcatggtgcaggggtaaaaactccggtggtacaggatggacccgcgtctgattagctggttggtgaggtaacggctcaccaaggcgacgatcagtagccggcttgagagagtgaacggccacattgggactgagacacggcccaaactcctacgggaggcagcagtggggaatattgcacaatgggggaaaccctgatgcagcgacgccgcgtgagtgaagaagtatctcggtatgtaaagctctatcagcagggaagaaaatgacggtacctgactaagaagccccggctaactacgtgccagcagccgcggtaatacgtagggggcaagcgttatccggaattactgggtgtaaagggtgcgtaggtggtatggcaagtcagaagtgaaaacccagggcttaactctgggactgcttttgaaactgtcagactggagtgcaggagaggtaagcggaattcctagtgtagcggtgaaatgcgtagatattaggaggaacatcagtggcgaaggcggcttactggactgaaactgacactgaggcacgaaagcgtggggagcaaacaggattagataccctggtagtccacgccgtaaacgatgaatactaggtgtcggggccgtagaggcttcggtgccgcagccaacgcagtaagtattccacctggggagtacgttcgcaagaatgaaactcaaaggaattgacggggacccgcacaagcggtggagcatgtggtttaattcgaagcaacgcgaagaaccttacctggtcttgacatccttctgaccggtccttaaccggacctttccttcgggacaggagtgacaggtggtgcatggttgtcgtcagctcgtgtcgtgagatgttgggttaagtcccgcaacgagcgcaacccctatctttagtagccagcaatataaggtgggcactctagagagactgccagggataacctgggaggaaggtggggacgacgtcaaatcatcatgccccttatgaccagggctacccccgtgctacaatgggcttaaaccaaggggaaa

SEQ ID NO: 2 - DNA, 1232 bp, unidentified
  source 1..1232: mol_type = genomic DNA
ggaattggcgggccgctacacatgcagtcgaacggcacccctctccggagggaagcgagtggcgaacggctgagtaacacgtggagaacctgccccctcccccgggatagccgcccgaaaggacgggtaataccggatacccccgggcgccgcatggcgcccgggctaaagccccgacgggaggggatggctccgcggcccatcaggtagacggcggggtgacggcccaccgtgccgacaacgggtagccgggttgagagaccgaccggccagattgggactgagacacggcccagactcctacgggaggcagcagtggggaatcttgcgcaatggggggaaccctgacgcagcgacgccgcgtgcgggacggaggccttcgggtcgtaaaccgctttcagcagggaagagtcaagactgtacctgcagaagaagccccggctaactacgtgccagcagccgcggtaatacgtagggggcgagcgttatccggattcattgggcgtaaagcgcgcgtaggcggcccggcaggccgggggtcgaagcggggggctcaaccccccgaagcccccggaacctccgcggcttgggtccggtaggggagggtggaacacccggtgtagcggtggaatgcgcagatatcgggtggaacaccggtggcgaaggcggccctctgggccgagaccgacgctgaggcgcgaaagctgggggagcgaacaggattagataccctggtagtcccagccgtaaacgatggacgctaggtgtggggggacgatccccccgtgccgcagccaacgcattaagcgtcccgcctggggagtacggccgcaaggctaaaactcaaaggaattgacgggggcccgcacaagcagcggagcatgtggcttaattcgaagcaacgcgaagaaccttaccagggcttgacatatgggtgaagcgggggagaccccgtggccgagaggagcccatacaggtggtgcatggctgtcgtcagctcgtgtcgtgagatgttgggttaagtcccgcaacgagcgcaacccccgccgcgtgttgccatcgggtgatgccgggaacccacgcgggaccgccgccgtcaaggcggaaggagggcggggacgacgtcaagtcatcatgccccttatgccctgggctgcacacgtgctacaatgggccggtacaaagggatgccccccccgcgagggggaaccggatcccggaaagccggcccc

SEQ ID NO: 3 - DNA, 1240 bp, unidentified
  source 1..1240: mol_type = genomic DNA
tgaatggccgcgtgcttacacatgcagtcgaacgggaatatatcttctattgagacttcggtggatttagattctaatttctagtggcggacgggtgagtaacgcgtgggtaacctgccttatacagggggataacagtcagaaatggctgctaataccgcataagcgcacagagctgcatggctcagtgtgaaaaactccggtggtataagatggacccgcgttggattagcttgttggtggggtaacggcccaccaaggcgacgatccatagccggcctgagagggtgaacggccacattgggactgagacacggcccagactcctacgggaggcagcagtggggaatattgcacaatgggggaaaccctgatgcagcgacgccgcgtgaaggaagaagtatctcggtatgtaaacttctatcagcagggaagatagtgacggtacctgactaagaagccccggctaactacgtgccagcagccgcggtaatacgtagggggcaagcgttatccggatttactgggtgtaaagggagcgtagacggtgtggcaagtctgatgtgaaaggcatgggctcaacctgtggactgcattggaaactgtcatacttgagtgccggaggggtaagcggaattcctagtgtagcggtgaaatgcgtagatattaggaggaacaccagtggcgaaggcggcttactggacggtaactgacgttgaggctcgaaagcgtggggagcaaacaggattagataccctggtagtccacgccgtaaacgatgaatactaggtgtcggggagcatagctcttcggtgccgtcgcaaacgcagtaagtattccacctggggagtacgttcgcaagaatgaaactcaaaggaattgacggggacccgcacaagcggtggagcatgtggtttaattcgaagcaacgcgaagaaccttaccaagtcttgacatccgtctgaccgatccttaatcggatctttccttcgggacaggcgagacaggtggtgcatggttgtcgtcagctcgtgtcgtgagatgttgggttaagtcccgcaacgagcgcaacccctatcctcagtagccagcatttaaggtgggcactctggggagactgccagggataacctggaggaaggcggggatgacgtcaaatcatcatgccccttatgatttgggctaccacctgctacaatggggtaaccaagggagacggaaatggtggaaagggggcaat

SEQ ID NO: 4 - DNA, 1244 bp, unidentified
  source 1..1244: mol_type = genomic DNA
gggaatttgcggcgtgcttacacatgcaagtcgaacgggatccatcaggctttgcttggtggtgagagtggcgaacgggtgagtaatgcgtgaccgacctgccccatacaccggaatagctcctggaaacgggtggtaatgccggatgctccagttgatcgcatggtcttctgggaaagctttcgcggtatgggatggggtcgcgtcctatcagcttgacggcggggtaacggcccaccgtggcttcgacgggtagccggcctgagagggcgaccggccacattgggactgagatacggcccagactcctacgggaggcagcagtggggaatattgcacaatgggcgcaagcctgatgcagcgacgccgcgtgagggatggaggccttcgggttgtaaacctcttttatcggggagcaagcgagagtgagtttacccgttgaataagcaccggctaactacgtgccagcagccgcggtaatacgtagggtgcaagcgttatccggaattattgggcgtaaagggctcgtaggcggttcgtcgcgtccggtgtgaaagtccatcgcttaacggtggatccgcgccgggtacgggcgggcttgagtgcggtaggggagactggaattcccggtgtaacggtggaatgtgtagatatcgggaagaacaccaatggcgaaggcaggtctctgggccgttactgacgctgaggagcgaaagcgtggggagcgaacaggattagataccctggtagtccacgccgtaaacggtggatgctggatgtggggcccgttccacgggttccgtgtcggagctaacgcgttaagcatcccgcctggggagtacggccgcaaggctaaaactcaaagaaattgacgggggcccgcacaagcggcggagcatgcggattaattcgatgcaacgcgaagaaccttacctgggcttgacatgttcccgacggtcgtagagatacggcttcccttcggggcgggttcacaggtggtgcatggtcgtcgtcagctcgtgtcgtgagatgttgggttaagtcccgcaacgagcgcaaccctcgccccgtgttgccagcggattatgccgggaactcacgggggaccgccggggtaactcggaggaaggtggggatgacgtcagatcatcatgccccttacgtccagggcttccgcatgctacaatggccggtacaacgggatgcaacccgggaacccggaacggatccctgaaaaccggttt